European Patent Application EP 4 115 889 A1, published January 11, 2023. Title: Therapeutic drug for tooth regeneration comprising RNA molecule targeting USAG-1. Applicant: Kyoto University UNIVERSITY OF FUKUI AICHI PREFECTURE. The sequence listing filed with the application follows.

SEQUENCE LISTING (10 sequences)

SEQ ID NO: 1 - RNA, 25 nt, Artificial
  siRNA
ccucuaacauguauaaagggugcaa

SEQ ID NO: 2 - RNA, 25 nt, Artificial
  siRNA
uugcacccuuuauacauguuagagg

SEQ ID NO: 3 - RNA, 25 nt, Artificial
  siRNA
auuugucaauguuauuauuuaauga

SEQ ID NO: 4 - RNA, 25 nt, Artificial
  siRNA
ucauuaaauaauaacauugacaaau

SEQ ID NO: 5 - RNA, 25 nt, Artificial
  siRNA
ucaguagcacuggacuggaucgaaa

SEQ ID NO: 6 - RNA, 25 nt, Artificial
  siRNA
uuucgauccaguccagugcuacuga

SEQ ID NO: 7 - RNA, 25 nt, Artificial
  siRNA
caagugucucaagauguaaugagua

SEQ ID NO: 8 - RNA, 25 nt, Artificial
  siRNA
uacucauuacaucuugagacacuug

SEQ ID NO: 9 - RNA, 25 nt, Artificial
  siRNA
ggccacuuaccacagagcuauuaaa

SEQ ID NO: 10 - RNA, 25 nt, Artificial
  siRNA
uuuaauagcucugugguaaguggcc